European Patent Application EP 4 600 344 A1, published August 13, 2025. Title: Microbial strain, protein, method for producing gallic acid using microbial strain or protein. Applicant: 国立大学法人筑波大学. The sequence listing filed with the application follows.

SEQUENCE LISTING (42 sequences)

SEQ ID NO: 1 - DNA, 1209 bp, Hylemonella gracilis
  source 1..1209: mol_type = genomic DNA
atgtcttatcccacaagaactcaggtcgctatcatcggtgccggacctagtggcctcatgctgggcgctctgctgcacaaagcggggattgacaccgtagtcctcgaacggcagtctggcgattatgtgcttggacgcattagagccggcgttttggaacaagtgacgatggaccttatggacgagataggagtaggggccagaatgcaccaggaaggtctggtgcatggaggcttcgatatgctctttcaggggcaacgccataggattgacatgaatcggctgactggaggtcagaatgtgatggtttatgggcagacagaggtgacaagagacttgatggatgcaaggcagcaagcgggactgaccaccatctacgaagccgctaatgtggccatacacgactttggcagcgggaaacctcgagtgacttatgagaaagacggcaaaacccacgaactgcagtgcgacttcattgcaggctgcgacggctttcacggcgtctgtcgggataccgtgaagaagtccgccagtgccagtgcaatccgcgagtacgaaaaggtgtacaacttcgggtggctgggtttgctgtccgatacccctccggtccaccacgaactcatctacgtaaacagcgagagaggcttcgccctgtgttcccagaggtctgcgacgaggagccggtattacctccaggtgccactgacagataaggtcgaacagtggtcagatcaggccttttgggatgagctcaaactgcgccttgacccacaagccagagagcatctggttaccggacccagcatagagaagagcatcgcacccctcaggtccttcgtgacagagccactgcggtttgggcgactgttccttgctggcgatgctgggcacatcgttcctccgactggcgcaaagggattgaacctggccgccaccgacgtcaagtatctcagcgctgcactgaccgagttctaccagggaaagtccgaggctgggatcaaccactactcagaacgctgcctgaagaggatttggcgagctgagaggttctcatggtggtttacgtccctgatgcatcggttccccgaaaatggcgagattgggcagaaattgcaagaggccgaactggactacatcgtccattccgagactggtgccaggtctgtggcggaaaactacgtgggactgcccctcgacttcggtgcctaa

SEQ ID NO: 2 - DNA, 48 bp, Hylemonella gracilis
  source 1..48: mol_type = other DNA
atcaccacagccaggatccgaattcaagctatcccacaagaactcagg

SEQ ID NO: 3 - DNA, 43 bp, Hylemonella gracilis
  source 1..43: mol_type = other DNA
ttaagcattatgcggccgcaagcttaggcaccgaagtcgaggg

SEQ ID NO: 4 - DNA, 1176 bp, Hydrogenophaga sp.
  source 1..1176: mol_type = genomic DNA
atgcgcacccaggttggtatcatcggcgccggcccggccggattgatgctcgcgcacatgcttcaccttgagggcattgaatctgtaattatcgaacgtagcaagcgcgagcatgtacaaaatcgtttgcgcgccggcgttctggaacagggcacggtagaaatgatgcgtgaactcggcttgggagaacgcatcggacagctgggattggagcaacatcgtatcgactttcgttttggaggagaatcccatcccattgatttccacgaagctaccggcggacggtcggcttgggtatatccccaacacgaagtggtcaaagatctgatggctgcacgtaccgctgccggtgcccagatgctcttcgaaacgcctgttactgctattgaaggaattgacggcacccgcccagtagttcgttttgaaaaggacggagtcgcgggagaactgcactgtgatttcgttgttggttgtgacggttttcgtggtatttcacgtcgtgctatcccagcccgtgaaggacaagtgcacgatcggatctatccgtttggttggctgggtatcctcgccgaggctccacccgcgactaatgaagtaacctggggctgtcacgaggacggctttgctatgatgtccattcggacgcctagcgtaacccgtttgtatctgcagtgcgaacctgatgaaaacccggaccattggtccgacgaccgtatttggtcggcactgcataagcggttggacgtgcctggattgccaccaatcaacgaaggtcgcattacccagaaaggcgtaacggccatgcgttcttttttgtttgagcccatgcaacacggtcgtctgtttctggccggtgacgccgctcacatcgtccctccgaccggcgccaagggactgaactctgcgatggcagacgtaaaagtcctcgcccgcgcgttggagcaacactaccaacgtggatcccaggaccttttggctcgttattcaaagacttgtctgaagcgcatgtggttggttcaacggttctcggccggactctgcacgatggtacatagcttcgcaggcgattcttctttcgttcgtcgccttcagcgcgctgacttggattacatgaccggcacgaccgcgggccgcttgcagttctcagagaatttcacgggcttgcccatcgactaa

SEQ ID NO: 5 - DNA, 43 bp, Hydrogenophaga sp.
  source 1..43: mol_type = other DNA
atcaccacagccaggatccgaattcgcggacccaggtcggcat

SEQ ID NO: 6 - DNA, 61 bp, Hydrogenophaga sp.
  source 1..61: mol_type = other DNA
ttaagcattatgcggccgcaagcttattcaatcggaagtccagtgaaattctctgaaaacg

SEQ ID NO: 7 - DNA, 1176 bp, Polaromonas sp.
  source 1..1176: mol_type = genomic DNA
atgcggacccaggtcggcatcgtgggtgcgggtcctgccggattgatgttgtcacacatgctccaccttgaaggtatcgaatcagtgatcatcgaacgcgcatcacgcgagcatgtacaaagccgccttcgggccggtgtacttgagcatggcaccgttgacatgctgcgcgagttgggcttgggtgagcgcattggcaagattggcttggagcagcatgctattgattttcggtttggaggcgagtcccatcgcttggactttcaccaagcgacgaatggacggtcggcatgggtgtaccctcagcatgagttggtgactgatttgatgaatgcacgtatgcaagctggtgctgagattctcttcgaaactcccgtaactcggattgacggactgcataccagcaaaccaactgttcacttcgagcaaggaggcgagccgcgtgagctcgtctgtgacttcgtggtaggttgtgacggctttcgtggtgtatgtcgtgatgctattcctgataccgtacttaaaacttacgatcgtgtgtaccccttcggctggctgggtattttggctgaagcaccggccccgactcgcgaaatcacttggggctgccacgaagaaggatttgccatgctctctatccgttcgccgagcgtgacccgtttgtatctccagtgcgaacctgatgatgatcctgatcattggagcgacgaccatatctgggcagagctgcacaagcggcttgatgttcccggcatgccccccgttaatgagggaaagattatgcaaaaaggtgtgaccgccatgcgctcgtttttggcagagcctatgcaatatggcaagcttttccttgcaggagacgccgcccacattgtgcccccaaccggagctaaaggtctcaattccgctatggcggatgtcaaagtgcttggtcgtggcttggctgaaaagtaccggcgtggtgctgatcaccttttggaacgttattcccaaatctgtctcaagcgcatgtggttggtacaacgtttttccgcgggcttgtgcacgatggtgcaccaattccccggtgataacgcttttgtgcggcgcttgcaacgggctgaccttgattacatgaccggaacggcggcgggacgtctcgcgttttcagagaatttcactggacttccgattgaataa

SEQ ID NO: 8 - DNA, 44 bp, Polaromonas sp.
  source 1..44: mol_type = other DNA
atcaccacagccaggatccgaattcgcgcacccaggttggtatc

SEQ ID NO: 9 - DNA, 41 bp, Polaromonas sp.
  source 1..41: mol_type = other DNA
ttaagcattatgcggccgcaagcttagtcgatgggcaagcc

SEQ ID NO: 10 - DNA, 27 bp, Hylemonella gracilis
  source 1..27: mol_type = other DNA
ctgtggcggaaaactacgtgggactgc

SEQ ID NO: 11 - DNA, 27 bp, Hylemonella gracilis
  source 1..27: mol_type = other DNA
gcagtcccacgaagttttccgccacag

SEQ ID NO: 12 - DNA, 27 bp, Hylemonella gracilis
  source 1..27: mol_type = other DNA
catcgttcctccggctggcgcaaaggg

SEQ ID NO: 13 - DNA, 27 bp, Hylemonella gracilis
  source 1..27: mol_type = other DNA
ccctttgcgccagccggaggaacgatg

SEQ ID NO: 14 - DNA, 1185 bp, Pseudomonas aeruginosa
  source 1..1185: mol_type = genomic DNA
atgaaaacacaggtagccatcattggtgcgggtccaagtgggttgttgctcggccagttactccacaaagcaggcatcgataacgtgattctggagcgtcaaacgccggattacgtactgggacgcattcgcgcgggagtgctggaacaaggtatggttgatctgctgcgtgaagcgggagtagatcgccggatggcgcgcgacggcttagtgcatgaaggtgtcgagatcgctttcgctgggcaacgccgtcggatcgacctgaaacgcctgtctggcggtaaaacggtgaccgtgtatggccagacagaagtgacgcgtgacctgatggaggcacgtgaagcctgtggcgctacgaccgtttatcaggccgcggaagtccgcttacacgatttgcagggtgaacgtccgtatgtcaccttcgaacgggatggggaacgcctgcgcttggactgcgactatattgctggttgcgatggctttcatggcatttcacgtcagagcattccggcagaacgcttaaaagtgttcgaacgtgtctacccttttggttggttaggcctgcttgccgatactccacccgtttcgcacgaactgatctacgcaaatcatccgcgtggctttgccttgtgctcccaacgttccgcgacgcgctctcgttattacgtgcaagttccactcagtgagaaagttgaggattggagcgatgaacgcttctggaccgaactcaaggcacgcttacccagtgaggtagccgaaaagctggtgactggcccgtcacttgaaaagagcattgcaccgttgcgctcgtttgttgtcgaacctatgcagcatggccgcctgtttctggcgggagatgccgcgcacattgttccgcctactggcgcgaaagggctgaatctggcagcttcagacgtttctaccctctatcgcctgctgcttaaagcctatcgtgagggtcgtggggaactgctggaacgctattcggcgatctgtctgcgccgtatctggaaagcggaacgctttagctggtggatgaccagcgtgctgcatcggtttccggataccgacgccttcagccagcgcatccagcagaccgaactggagtactaccttggctccgaagctggtctggcgacaattgcggaaaactacgtcggtctgccgtatgaggagattgagtaa

SEQ ID NO: 15 - DNA, 22 bp, Pseudomonas aeruginosa
  source 1..22: mol_type = other DNA
ttcgtcggtctgccgtatgagg

SEQ ID NO: 16 - DNA, 21 bp, Pseudomonas aeruginosa
  source 1..21: mol_type = other DNA
gttttccgcaattgtcgccag

SEQ ID NO: 17 - DNA, 1188 bp, Corynebacterium glutamicum
  source 1..1188: mol_type = genomic DNA
atgaatcacgtacctgtggcaatcattggagctggccccgcgggtctgacgctggcccacctgctgcatcttcaaggcgtcgagagcattgtgttcgagtctcggacgcgcaaggatgtagaagagactgttcgtgctggaatcttggaacaaggcacgctcaatttgatgcgtgaaaccggtgtcggagcacgtatggaagccgaggctgaccatgacgaggcaatcgacatctctatcaacaatgagcgcacgcgcatcccgcttaccgagttgacgggccacaaagtagctatttacccacagcatgaatatctgaaggatttcatcgcaaagcgcatcgaggacggtggagaactcttgtttaccacgactgtagacagcgttgaaaactacgaaggagacctggctaaggttacgtataccgaagcagacggatcaagcactactattaccgctgactacgttatcgccgcggacggctcgaactcgccttatcgcaagctcattaccgaagatggcggtgtacgtgcgcgccatgaatatccatacgcttggttcggtatcctcgtagaggcccccaaaacccaaaaggagctgatttatgcgacgcacccggaaggcttcgccctgatcagcacgcgtactgacgaaatccagcggtattatctgcaatgcaatccagatgatacccccgacatgtggccggacgatcgcatttgggagcagttgcaccttcgtgccgatagccctggaattactgtgtccgagggacggattttcgacaaagcggttctgcgtttctgttccgcggtcacggagcctatgcagaaaggccgcctgtttttggcgggagatgcggctcataccgtaccgcctacgggtgcaaaaggcctcaatctggcggtagctgatgtatccgtcctggcacccgcgttggttcgtgcattgaagaagaaggataccggtcttctggattcctacaccagcctggcagttccacgcatctggaaagctcaacacttttcttattggatgtcgtcaatgctccacgccgtgcccggagaggatcacttcgcaacgcaacgccgtttcgccgaacttcgttctgtcctggagtctcagagcggacaacgttacctcgctgagcaatacgttggccgggatctcccgcggtttgaagtgtaa

SEQ ID NO: 18 - DNA, 43 bp, Corynebacterium glutamicum
  source 1..43: mol_type = other DNA
atcaccacagccaggatccgaattcaaatcacgtacctgtggc

SEQ ID NO: 19 - DNA, 41 bp, Corynebacterium glutamicum
  source 1..41: mol_type = other DNA
ttaagcattatgcggccgcaagcttacacttcaaaccgcgg

SEQ ID NO: 20 - protein, 402 aa, Hylemonella gracilis
MSYPTRTQVAIIGAGPSGLMLGALLHKAGIDTVVLERQSGDYVLGRIRAGVLEQVTMDLMDEIGVGARMHQEGLVHGGFDMLFQGQRHRIDMNRLTGGQNVMVYGQTEVTRDLMDARQQAGLTTIYEAANVAIHDFGSGKPRVTYEKDGKTHELQCDFIAGCDGFHGVCRDTVKKSASASAIREYEKVYNFGWLGLLSDTPPVHHELIYVNSERGFALCSQRSATRSRYYLQVPLTDKVEQWSDQAFWDELKLRLDPQAREHLVTGPSIEKSIAPLRSFVTEPLRFGRLFLAGDAGHIVPPAGAKGLNLAATDVKYLSAALTEFYQGKSEAGINHYSERCLKRIWRAERFSWWFTSLMHRFPENGEIGQKLQEAELDYIVHSETGARSVAENFVGLPLDFGA

SEQ ID NO: 21 - protein, 391 aa, Hydrogenophaga sp.
MRTQVGIIGAGPAGLMLAHMLHLEGIESVIIERSKREHVQNRLRAGVLEQGTVEMMRELGLGERIGQLGLEQHRIDFRFGGESHPIDFHEATGGRSAWVYPQHEVVKDLMAARTAAGAQMLFETPVTAIEGIDGTRPVVRFEKDGVAGELHCDFVVGCDGFRGISRRAIPAREGQVHDRIYPFGWLGILAEAPPATNEVTWGCHEDGFAMMSIRTPSVTRLYLQCEPDENPDHWSDDRIWSALHKRLDVPGLPPINEGRITQKGVTAMRSFLFEPMQHGRLFLAGDAAHIVPPTGAKGLNSAMADVKVLARALEQHYQRGSQDLLARYSKTCLKRMWLVQRFSAGLCTMVHSFAGDSSFVRRLQRADLDYMTGTTAGRLQFSENFTGLPID

SEQ ID NO: 22 - protein, 391 aa, Polaromonas sp.
MRTQVGIVGAGPAGLMLSHMLHLEGIESVIIERASREHVQSRLRAGVLEHGTVDMLRELGLGERIGKIGLEQHAIDFRFGGESHRLDFHQATNGRSAWVYPQHELVTDLMNARMQAGAEILFETPVTRIDGLHTSKPTVHFEQGGEPRELVCDFVVGCDGFRGVCRDAIPDTVLKTYDRVYPFGWLGILAEAPAPTREITWGCHEEGFAMLSIRSPSVTRLYLQCEPDDDPDHWSDDHIWAELHKRLDVPGMPPVNEGKIMQKGVTAMRSFLAEPMQYGKLFLAGDAAHIVPPTGAKGLNSAMADVKVLGRGLAEKYRRGADHLLERYSQICLKRMWLVQRFSAGLCTMVHQFPGDNAFVRRLQRADLDYMTGTAAGRLAFSENFTGLPIE

SEQ ID NO: 23 - protein, 397 aa, Limnohabitans sp.
MSTTRTQVAIVGAGPSGLLLGQLLFKAGIDAIIVERQSPDYVLSRIRAGVLEQVTMDLLDEAGVGQRMHKEGLVHTGFDLLFKGARHRIDMDHLTGGKKVIVYGQTEVTRDLMDTRQAEGLPTVYEAGNVQVHDFDSQKPRVTYEKNGQLHTIECDFIAGCDGFHGVCRASAPKNAIKEYEKVYPFGWLGVLSDTPPVHHELIYANSTRGFALCSQRSATRSRYYLQVPTTDKVEQWSDDAFWAELRNRLDPEAREHLVTGPSIEKSIAPLRSFVTEPMRFGRMFLAGDAAHIVPPTGAKGLNLAATDVKYLSTAFIEFYADQTEAGIDAYSERCLRRVWRAERFSWWFTSLMHHFPENGDIGQKFQDAELDYLIHSEAGSRTMAENYVGLPLNFGE

SEQ ID NO: 24 - protein, 391 aa, Rhodoferax sedimins
MRTQVGIVGAGPAGLMLSHMLHLEGIESVIIERASREHVQSRLRAGVLEHGTVDMLKELGLGERISTLGLEQHAIDFRFGGESHRLDFHQATNGRRTWVYPQHEVVTDLMKARMQAGAQILFETSVTRIEGLQTRKPTIHFEQGGEPRELQCDFIVGCDGFRGVCRDAIPDSVLKIYDRVYPFGWLGILAEAPAPTNEITWGCHEDGFAMLSIRSPSVTRLYLQCEPNEDADRWSDGRIWAELHKRLDVPGMPPVNEGKITQKGVTAMRSFLAEPMQYGRLFLAGDAAHIVPPTGAKGLNSSMADVKVLGRGLVEQYKRGVADILDRYSQICLKRMWLVQRFSAGLCTMVHQIPGDNAFVRRLQRADLDYMTGTVAGRLAFSENFTGLPIE

SEQ ID NO: 25 - protein, 391 aa, Xylophilus ampelinus; identical to SEQ ID NO: 24

SEQ ID NO: 26 - protein, 390 aa, Ramlibacter henchirensis
MRTQVGIVGAGPAGLMLAQILHLQGIDSVLIERASQEHVRSRLRAGVLEQGTVEMMREFGVGERVMKVGLRQRAIDFRFNGESHPIDFESVCGRNTWVYPQHEVVSDLMAARERSGLPVVYDAPVSRIEGLDGGRPVIHYERDGEPLRLECDYVAGCDGFRGISRSWIPADRLKVYDRIYPFGWLGILADAKPAIQDITWGCHEDGFAMMSIRSPTVTRLYLQCEPDENPDDWPDDRIWAELHKRLDVPGLPRLEEGRITQKGVTAMRSFLAEPMQYGRLFLAGDAAHIVPPTGAKGLNSALADVKVLARALTEQYRNENGQWLERYSDICLKRMWLVQRFSSGLCTMTHQFRGDEPFVRRLQRADLEYMTMHAPGRLEFSENFTGLPVE

SEQ ID NO: 27 - protein, 374 aa, Comamonas phosphati
MSHMLHLAGIESVVLERAGREHVRTRLRAGVLEQGVVEMLRELGLGERLDQLALKQSALDFRFDGASRRIDFEAEIGRNVWVYPQHEVVTDLMNARQKAGAAIFYEAPVQRIDGLEGERPVLHFEHQGESCRLECDYVAGCDGFRGVSRSAIPADKLKVFDRIYPFGWLGILAEAPAATNEIVWGCHDGGFAMQSIRSPSVTRLYLQCAPDENPDHWSDDRIWSELHKRLDVEGMPPVNEGRVTQKGVTAMRSFLAEPMQWGRLFLAGDAAHIVPPTGAKGLNSALADIKVLARALVAHYREGADAHLARYSDTCLRRMWLVQRFSAGLCTMTHQFPGQNPFVQRLQRTDLDYMTGTRAGRLQFSENFTGLPVE

SEQ ID NO: 28 - protein, 394 aa, Pseudomonas aeruginosa
MKTQVAIIGAGPSGLLLGQLLHKAGIDNVILERQTPDYVLGRIRAGVLEQGMVDLLREAGVDRRMARDGLVHEGVEIAFAGQRRRIDLKRLSGGKTVTVYGQTEVTRDLMEAREACGATTVYQAAEVRLHDLQGERPYVTFERDGERLRLDCDYIAGCDGFHGISRQSIPAERLKVFERVYPFGWLGLLADTPPVSHELIYANHPRGFALCSQRSATRSRYYVQVPLSEKVEDWSDERFWTELKARLPSEVAEKLVTGPSLEKSIAPLRSFVVEPMQHGRLFLAGDAAHIVPPTGAKGLNLAASDVSTLYRLLLKAYREGRGELLERYSAICLRRIWKAERFSWWMTSVLHRFPDTDAFSQRIQQTELEYYLGSEAGLATIAENYVGLPYEEIE

SEQ ID NO: 29 - protein, 395 aa, Corynebacterium glutamicum
MNHVPVAIIGAGPAGLTLAHLLHLQGVESIVFESRTRKDVEETVRAGILEQGTLNLMRETGVGARMEAEADHDEAIDISINNERTRIPLTELTGHKVAIYPQHEYLKDFIAKRIEDGGELLFTTTVDSVENYEGDLAKVTYTEADGSSTTITADYVIAADGSNSPYRKLITEDGGVRARHEYPYAWFGILVEAPKTQKELIYATHPEGFALISTRTDEIQRYYLQCNPDDTPDMWPDDRIWEQLHLRADSPGITVSEGRIFDKAVLRFRSAVTEPMQKGRLFLAGDAAHTVPPTGAKGLNLAVADVSVLAPALVRALKKKDTGLLDSYTSLAVPRIWKAQHFSYWMSSMLHAVPGEDHFATQRRFAELRSVLESQSGQRYLAEQYVGRDLPRFEV

SEQ ID NO: 30 - protein, 408 aa, Corynebacterium ammoniagenes
MGTPTNSDSSHTPVAIIGAGPAGLMLSHLLHLEGVESVVIEKQSREEVESTVRAGILEQGTIDLLRKTGVGERLDREAEIDEGISISIAGESHRIDFAKYTGKQVAVYPQHEVLIDLIAKRLSDDGELWFDTEVVSIADHESDNPKVHYRTADGTEGVLSADFVVGADGSKSLARKLITDDGGLRMKHEYPFAWFGIMVNAPQTAPEVIYATHPEGFALISTRSENVQRYYLQCNPDDTPDMWSDDRIWEQLHLRADSDTVTVSEGEITDKAVLRFRSAVTDPMQRGRLFIAGDAAHTVPPTGAKGLNLAMADVCALAPSLVRAVKKSDTSLLDTYSERALPRVWKTQHFSYWMSSMLHSVPAENEMSTLFQTNRRLAELSTVVTSDAGRQLLAQQFVGWDFPSIEAL

SEQ ID NO: 31 - protein, 404 aa, Corynebacterium callunae
MNHIPVAIIGAGPAGLTLAHLLHLQGIESIVFEKRTRKEVEETVRAGILEQGTLNLMRETGVGARMEAEADHDEAIDISINGERIRIPLTEITGHKVAIYPQHEYLKDFIAKRLEDGGELLFSTTVDAVEGTGGTGGTEGFDNDKVKVVYTEADGSSTTISADYVIAADGSSSPYRKIITEGSGVRARHEYPYAWFGILVEAAKTQKEVIYATHPEGFALISTRTDTVQRYYLQCDPNDTPDMWSDDRIWEQLHLRADSPGITVSEGKIFDKAVLRFRSAVTEPMQKGRLFLAGDAAHTVPPTGAKGLNLAVADVSVLAPGLVRALKKKDSALLDDYTKLALPRVWKAQHFSYWMSSMLHAVPDEDYFATQRRFAELHSVLGSEAGQRYLAEQFVGRDLPRFEV

SEQ ID NO: 32 - protein, 399 aa, Corynebacterium efficiens
MNHVPVAIIGAGPAGLTLAHLLHLQGIESVVFESRSRQDVEETVRAGILEQGTLNLMRETGVGERMEREADHDEAIDIAINNENIRIPLTELTGHKVAIYPQHEYLKDFIAKRIEDGGELLFETTVDSVENFEGDAQENKATITYTGVDGTTRQLTADYVVAADGSNSPYRKIITDDGGIRARHEYPYAWFGILVEAPKTQKEVIYATHPEGFALISTRTDTVQRYYLQCDPNDTPEMWSDDRIWEQLHLRADSPGITVSEGKIFDKAVLRFRSAVTEPMQKGRLFIAGDAAHTVPPTGAKGLNLAVADVSVLAPGLTRAIKRNDTGLLDDYTRLTVPRIWKAQHFSYWMSSMLHAVPGEDHFATQRRFAELRSVLESEAGQRYLAEQFVGRDLPRFDY

SEQ ID NO: 33 - DNA, 2241 bp, Corynebacterium glutamicum
  source 1..2241: mol_type = genomic DNA
atgcgttttgatctccattctgtagttatttccacattggttttcgctgcggttgctttggtatggcgcttgttttttgtcggtggttggcttgtacgtcggcgtaaagcacgtatccgcaggcagacgctcgcggatgaagagcgggcagaaaatgctgaggtatctgcaggggagcctgccgaatcgagcacaaacgaagcagccgaatctgaatctgaaacctcggagcgtcgcggaatctggcgcgtgatctttgattacatgcgcgacggtggcatcttggatcaccgttggctgctgcctgccgcaggtgctatcactggtgcgtggctgatcattgatcgtgccgttgatctgctcttgagcaccgagcatggtttgggcgatatcgtccaaggctgggatgtccattggcatgcttcgactgtccgttttatagatgagaccggcattgcgtcatccacgatgatggggcagctgcgcaatattgaaacgcagcaagatctgttctacccaagcgcatggcatgctggtgcatgggtgctgtcggatgtcggaaatctgacgattgttgaagccaccaacctcactggcattgtgctgtccggattgttgctgccgttagctgttgcactgattgcatggcggatgatcaacaatcgtggactgaccgcgcagattggtgcgggctttgctggactgatcaccattgcctctccggtactgttctgggttggtaactacgtgggtgcgtggccttatgttgctgcgatcggtgcttcaggtgtggtgcttgcgctgtttatgtccactccgtctgtgccggtaagaatctttgccgcagcattggcgttcatgggtatgttccagctgcatccagccccatccaccatcgtgatcatggtgttgctgctgtggtggctgctcaaactcgtggtggttccaagccagaaagtgaagggctggaaggcgggcatcggtatccgtttgaaggatgtcggcatcctggccatcacgggcatcatcggtgtgctcttcatgctgcctcaggtgatttcaggttccgaacaaaccgaagatgtgctgtcatattctgctgaggaacaagtcacccgcagcgagtcctggttggtgtctattttcatggagacccgccatgttgatttcttcggaaatattgacatcgtcccagtgctggtattcgcagcaatcggtggcgtggttgctttggtgtggcgcggaaacttgtgggcgccggtgttttacttcgccagcgttgcgttgaccgctaactcgctgaagccttttgaagagccgtggggtgattggctcaacatcgtgggcggtctgcattactccacaggacaccgtttgatcatgcctgtcgccatgttcacttttgctgccgcaggtatcggcgctgccgcagtgatccgtttgatctgcttgggaccaataaagaagttcaccactgtttccggtgttgtttctgtggtgatggctcttgttgtggctgtgccattgcagacttgggcgaaggattttgtagaggaaggatccgaaaccacaatccttgcgccacacaatgatgaacgtatggtgagcaacaacgacttggctgcctgggactggttaatccaacagccaggtggagctgacatgaacatcatgggtgaccccgcagatggtaacggctggatgtatgcctacaacggcttgcactccgtggcccgccactatgcatggccagcagcaggcgaaggctctgccaccgcgatgctgttctggtggcctcaacttctaggtgtgggcaccgatgaaaacccagatcaagtcaacgatgtggatcaggctgctcgtgatctcaacgtcggctacttcatgatcagtccgtggacgttctgggatttccagatccccaacttccgccagatcgatctgctgtggcaaaccccaggcgtgacaccggtgtacaagaagggcgactcggtgatcttcgcagtcaacgatatgttcactgacgccgaactggatcagatgcgtgcacctggtaattctccagaaccactgccagagcttcctaccttgggcgagcttgggttggctgaaactgaagacgaggtagatcagacttattaccatcgtccaacggttcctgctggtgtgaactcagagatgccttcagccgaaactctgtatgcaccggatccaacgaagccgcatacggtccctaactaa

SEQ ID NO: 34 - DNA, 26 bp, Corynebacterium glutamicum
  source 1..26: mol_type = other DNA
gagctcatgcgttttgatctccattc

SEQ ID NO: 35 - DNA, 33 bp, Corynebacterium glutamicum
  source 1..33: mol_type = other DNA
gagctcctctagattagttagggaccgtatgcg

SEQ ID NO: 36 - DNA, 125 bp, Escherichia coli
  source 1..125: mol_type = genomic DNA
ttcgatttattcaacaaagccacgttgtgtctcaaaatctctgatgttacattgcacaagataaaaatatatcatcatgaacaataaaactgtctgcttacataaacagtaatacaaggggtgtt

SEQ ID NO: 37 - DNA, 1209 bp, Hylemonella gracilis
  source 1..1209: mol_type = genomic DNA
atgtcttaccctacgcggacccaggtagctatcatcggcgcaggtccgtcaggcctgatgttgggcgctcttctccacaaggctggtattgatacggttgttctcgaacgtcagtccggcgattatgttttgggacgtatccgcgccggagtactcgaacaagtgactatggatctgatggatgagattggagtcggcgcccgtatgcaccaggagggcttggttcacggtggttttgacatgctgtttcaaggccaacggcatcgtattgatatgaatcggttgactggcggacaaaatgtaatggtctacggtcagaccgaagtcacgcgggatcttatggatgctcgccaacaagccggtttgaccacgatctacgaggctgcaaacgtggcgattcatgatttcggaagcggcaaacctcgggtcacgtacgagaaggacggtaagacccacgagttgcagtgtgactttattgcaggttgtgacggctttcacggcgtatgccgggacacggttaaaaagagcgcttctgcgtctgcgatccgggagtatgaaaaagtgtacaactttggctggctgggtctcttgtctgatacgccgccggttcatcatgagctgatctatgtaaattctgagcgtggtttcgcactgtgcagccagcgctctgcgacccgttctcgttactatcttcaggtgccccttaccgataaagtagaacaatggagcgaccaagctttctgggacgaactgaaactgcggcttgatcctcaagcccgtgaacatttggttaccggtccatcaattgaaaagtctatcgcaccgctccggtcattcgttaccgaacccctgcggtttggccgtctcttcctggccggcgatgcgggacacattgtcccacctgccggagccaagggacttaatctggcagccactgatgtgaagtacttgagcgcggccctcacggaattttatcagggaaaatccgaggctggcatcaaccactactctgaacgctgtctgaagcgtatctggcgtgcagaacggttttcctggtggtttacttcactcatgcatcgtttcccggagaacggagagatcggccagaagcttcaggaagcagagctcgattacattgtccactcggaaaccggagcgcgttcggttgccgaaaactttgttggactccctctggatttcggtgcataa

SEQ ID NO: 38 - DNA, 27 bp, Escherichia coli
  source 1..27: mol_type = other DNA
gagctcatgcgcacccaggttggtatc

SEQ ID NO: 39 - DNA, 26 bp, Hydrogenophaga sp.
  source 1..26: mol_type = other DNA
gtcgacttagtcgatgggcaagcccg

SEQ ID NO: 40 - DNA, 26 bp, Polaromonas sp.
  source 1..26: mol_type = other DNA
gtcgacttattcaatcggaagtccag

SEQ ID NO: 41 - DNA, 26 bp, Hylemonella gracilis
  source 1..26: mol_type = other DNA
gtcgacttaggcaccgaagtcgaggg

SEQ ID NO: 42 - DNA, 25 bp, Corynebacterium glutamicum
  source 1..25: mol_type = other DNA
gtcgacttacacttcaaaccgcggg